European Patent Application EP 4 438 610 A1, published October 2, 2024. Title: Compound, racemic body and salt thereof, composition, anti-inflammatory drug, therapeutic agent for dementia and therapeutic agent for Rett syndrome. Applicant: INSTITUTE OF RHEOLOGICAL FUNCTION OF FOOD CO., LTD. Application WO. The sequence listing filed with the application follows.

SEQUENCE LISTING (4 sequences)

SEQ ID NO: 1 - DNA, 20 bp, synthetic construct
  misc_feature 1..20: note = Forward primer for IL-1 beta
  source 1..20: mol_type = other DNA
aaaaaagcctcgtgctgtcg

SEQ ID NO: 2 - DNA, 21 bp, synthetic construct
  misc_feature 1..21: note = Reverse primer for IL-1 beta
  source 1..21: mol_type = other DNA
gtcgttgcttggttctccttg

SEQ ID NO: 3 - DNA, 18 bp, synthetic construct
  misc_feature 1..18: note = Forward primer for beta-actin
  source 1..18: mol_type = other DNA
cactgtgcccatctacga

SEQ ID NO: 4 - DNA, 18 bp, synthetic construct
  misc_feature 1..18: note = Reverse primer for beta-actin
  source 1..18: mol_type = other DNA
caggattccatacccaag